European Patent Application EP 4 588 940 A2, published July 23, 2025. Title: ANTIBODY-DRUG CONJUGATE COMPRISING ANTIBODY AGAINST HUMAN ROR1 AND USE FOR THE SAME. Applicant: LEGOCHEM BIOSCIENCES, INC. The sequence listing filed with the application follows.

SEQUENCE LISTING (106 sequences)

SEQ ID NO: 1 - protein, 5 aa, synthetic construct
  source 1..5: note = Heavy chain CDR1
SYDMS

SEQ ID NO: 2 - protein, 5 aa, synthetic construct
  source 1..5: note = Heavy chain CDR1
DYYMS

SEQ ID NO: 3 - protein, 5 aa, synthetic construct
  source 1..5: note = Heavy chain CDR1
NYDMS

SEQ ID NO: 4 - protein, 5 aa, synthetic construct
  source 1..5: note = Heavy chain CDR1
NYAMS

SEQ ID NO: 5 - protein, 5 aa, synthetic construct
  source 1..5: note = Heavy chain CDR1
DYDMS

SEQ ID NO: 6 - protein, 17 aa, synthetic construct
  source 1..17: note = Heavy chain CDR2
WISPDSGSIYYADSVKG

SEQ ID NO: 7 - protein, 17 aa, synthetic construct
  source 1..17: note = Heavy chain CDR2
SISPDGSNTYYADSVKG

SEQ ID NO: 8 - protein, 17 aa, synthetic construct
  source 1..17: note = Heavy chain CDR2
WISPGGGSKYYADSVKG

SEQ ID NO: 9 - protein, 17 aa, synthetic construct
  source 1..17: note = Heavy chain CDR2
AIYHSGSSKYYADSVKG

SEQ ID NO: 10 - protein, 17 aa, synthetic construct
  source 1..17: note = Heavy chain CDR2
GISHGSGNKYYADSVKG

SEQ ID NO: 11 - protein, 17 aa, synthetic construct
  source 1..17: note = Heavy chain CDR2
SISHNSGSTYYADSVKG

SEQ ID NO: 12 - protein, 17 aa, synthetic construct
  source 1..17: note = Heavy chain CDR2
VISPDGGSIYYADSVKG

SEQ ID NO: 13 - protein, 18 aa, synthetic construct
  source 1..18: note = Heavy chain CDR2
SISPSSGSSIYYADSVKG

SEQ ID NO: 14 - protein, 7 aa, synthetic construct
  source 1..7: note = Heavy chain CDR3
PTGRFDY

SEQ ID NO: 15 - protein, 7 aa, synthetic construct
  source 1..7: note = Heavy chain CDR3
NLRAFDY

SEQ ID NO: 16 - protein, 7 aa, synthetic construct
  source 1..7: note = Heavy chain CDR3
VNGRFDY

SEQ ID NO: 17 - protein, 12 aa, synthetic construct
  source 1..12: note = Heavy chain CDR3
GGNGAWDTGFDY

SEQ ID NO: 18 - protein, 18 aa, synthetic construct
  source 1..18: note = Heavy chain CDR3
RLSLRRRPSYYSDNAMDV

SEQ ID NO: 19 - protein, 18 aa, synthetic construct
  source 1..18: note = Heavy chain CDR3
FISARKSLGRSYSNGMDV

SEQ ID NO: 20 - protein, 18 aa, synthetic construct
  source 1..18: note = Heavy chain CDR3
DVVECNMNPCSYDNAMDV

SEQ ID NO: 21 - protein, 18 aa, synthetic construct
  source 1..18: note = Heavy chain CDR3
APGWCQAPSCYYDNAMDV

SEQ ID NO: 22 - protein, 13 aa, synthetic construct
  source 1..13: note = Light chain CDR1
SGSSSNIGNNNVN

SEQ ID NO: 23 - protein, 13 aa, synthetic construct
  source 1..13: note = Light chain CDR1
SGSSSNIGSNTVY

SEQ ID NO: 24 - protein, 13 aa, synthetic construct
  source 1..13: note = Light chain CDR1
SGSSSNIGNNNVS

SEQ ID NO: 25 - protein, 13 aa, synthetic construct
  source 1..13: note = Light chain CDR1
SGSSSNIGSNDVS

SEQ ID NO: 26 - protein, 13 aa, synthetic construct
  source 1..13: note = Light chain CDR1
TGSSSNIGNNAVN

SEQ ID NO: 27 - protein, 13 aa, synthetic construct
  source 1..13: note = Light chain CDR1
TGSSSNIGSNDVT

SEQ ID NO: 28 - protein, 13 aa, synthetic construct
  source 1..13: note = Light chain CDR1
SGSSSNIGSNYVS

SEQ ID NO: 29 - protein, 13 aa, synthetic construct
  source 1..13: note = Light chain CDR1
SGSSSNIGNNDVS

SEQ ID NO: 30 - protein, 7 aa, synthetic construct
  source 1..7: note = Light chain CDR2
YDNKRPS

SEQ ID NO: 31 - protein, 7 aa, synthetic construct
  source 1..7: note = Light chain CDR2
ANSQRPS

SEQ ID NO: 32 - protein, 7 aa, synthetic construct
  source 1..7: note = Light chain CDR2
ADSHRPS

SEQ ID NO: 33 - protein, 7 aa, synthetic construct
  source 1..7: note = Light chain CDR2
YDNNRPS

SEQ ID NO: 34 - protein, 7 aa, synthetic construct
  source 1..7: note = Light chain CDR2
YDSNRPS

SEQ ID NO: 35 - protein, 7 aa, synthetic construct
  source 1..7: note = Light chain CDR2
ADSKRPS

SEQ ID NO: 36 - protein, 7 aa, synthetic construct
  source 1..7: note = Light chain CDR2
DDSHRPS

SEQ ID NO: 37 - protein, 7 aa, synthetic construct
  source 1..7: note = Light chain CDR2
DDSQRPS

SEQ ID NO: 38 - protein, 11 aa, synthetic construct
  source 1..11: note = Light chain CDR3
GTWDASLSGYV

SEQ ID NO: 39 - protein, 11 aa, synthetic construct
  source 1..11: note = Light chain CDR3
GSWDYSLSGYV

SEQ ID NO: 40 - protein, 11 aa, synthetic construct
  source 1..11: note = Light chain CDR3
ATWDYSLSGYV

SEQ ID NO: 41 - protein, 11 aa, synthetic construct
  source 1..11: note = Light chain CDR3
GAWDDSLSGYV

SEQ ID NO: 42 - protein, 11 aa, synthetic construct
  source 1..11: note = Light chain CDR3
GTWDYSLSGYV

SEQ ID NO: 43 - protein, 116 aa, synthetic construct
  source 1..116: note = Heavy chain variable region
EVQLLESGGGLVQPGGSLRLSCAASGFTFSSYDMSWVRQAPGKGLEWVSWISPDSGSIYYADSVKGRFTISRDNSKNTLYLQMNSLRAEDTAVYYCARPTGRFDYWGQGTLVTVSS

SEQ ID NO: 44 - protein, 116 aa, synthetic construct
  source 1..116: note = Heavy chain variable region
EVQLLESGGGLVQPGGSLRLSCAASGFTFSDYYMSWVRQAPGKGLEWVSSISPDGSNTYYADSVKGRFTISRDNSKNTLYLQMNSLRAEDTAVYYCAKNLRAFDYWGQGTLVTVSS

SEQ ID NO: 45 - protein, 116 aa, synthetic construct
  source 1..116: note = Heavy chain variable region
EVQLLESGGGLVQPGGSLRLSCAASGFTFSSYDMSWVRQAPGKGLEWVSWISPGGGSKYYADSVKGRFTISRDNSKNTLYLQMNSLRAEDTAVYYCARVNGRFDYWGQGTLVTVSS

SEQ ID NO: 46 - protein, 121 aa, synthetic construct
  source 1..121: note = Heavy chain variable region
EVQLLESGGGLVQPGGSLRLSCAASGFTFSNYDMSWVRQAPGKGLEWVSAIYHSGSSKYYADSVKGRFTISRDNSKNTLYLQMNSLRAEDTAVYYCARGGNGAWDTGFDYWGQGTLVTVSS

SEQ ID NO: 47 - protein, 127 aa, synthetic construct
  source 1..127: note = Heavy chain variable region
EVQLLESGGGLVQPGGSLRLSCAASGFTFSSYDMSWVRQAPGKGLEWVSGISHGSGNKYYADSVKGRFTISRDNSKNTLYLQMNSLRAEDTAVYYCAKRLSLRRRPSYYSDNAMDVWGQGTLVTVSS

SEQ ID NO: 48 - protein, 127 aa, synthetic construct
  source 1..127: note = Heavy chain variable region
EVQLLESGGGLVQPGGSLRLSCAASGFTFSNYAMSWVRQAPGKGLEWVSSISHNSGSTYYADSVKGRFTISRDNSKNTLYLQMNSLRAEDTAVYYCAKFISARKSLGRSYSNGMDVWGQGTLVTVSS

SEQ ID NO: 49 - protein, 127 aa, synthetic construct
  source 1..127: note = Heavy chain variable region
EVQLLESGGGLVQPGGSLRLSCAASGFTFSDYDMSWVRQAPGKGLEWVSVISPDGGSIYYADSVKGRFTISRDNSKNTLYLQMNSLRAEDTAVYYCARDVVECNMNPCSYDNAMDVWGQGTLVTVSS

SEQ ID NO: 50 - protein, 128 aa, synthetic construct
  source 1..128: note = Heavy chain variable region
EVQLLESGGGLVQPGGSLRLSCAASGFTFSNYDMSWVRQAPGKGLEWVSSISPSSGSSIYYADSVKGRFTISRDNSKNTLYLQMNSLRAEDTAVYYCAKAPGWCQAPSCYYDNAMDVWGQGTLVTVSS

SEQ ID NO: 51 - protein, 111 aa, synthetic construct
  source 1..111: note = Light chain variable region
QSVLTQPPSASGTPGQRVTISCSGSSSNIGNNNVNWYQQLPGTAPKLLIYYDNKRPSGVPDRFSGSKSGTSASLAISGLRSEDEADYYCGTWDASLSGYVFGGGTKLTVLG

SEQ ID NO: 52 - protein, 111 aa, synthetic construct
  source 1..111: note = Light chain variable region
QSVLTQPPPASGTPGQRVTISCSGSSSNIGSNTVYWYQQLPGTAPKLLIYANSQRPSGVPDRFSGSKSGTSASLAISGLRSEDEADYYCGSWDYSLSGYVFGGGTKLTVLG

SEQ ID NO: 53 - protein, 111 aa, synthetic construct
  source 1..111: note = Light chain variable region
QSVLTQPPSASGTPGQRVTISCSGSSSNIGNNNVSWYQQLPGTAPKLLIYADSHRPSGVPDRFSGSKSGTSASLAISGLRSEDEADYYCATWDYSLSGYVFGGGTKLTVLG

SEQ ID NO: 54 - protein, 111 aa, synthetic construct
  source 1..111: note = Light chain variable region
QSVLTQPPSASGTPGQRVTISCSGSSSNIGSNDVSWYQQLPGTAPKLLIYYDNNRPSGVPDRFSGSKSGTSASLAISGLRSEDEADYYCGAWDDSLSGYVFGGGTKLTVLG

SEQ ID NO: 55 - protein, 111 aa, synthetic construct
  source 1..111: note = Light chain variable region
QSVLTQPPSASGTPGQRVTISCTGSSSNIGNNAVNWYQQLPGTAPKLLIYYDSNRPSGVPDRFSGSKSGTSASLAISGLRSEDEADYYCGAWDDSLSGYVFGGGTKLTVLG

SEQ ID NO: 56 - protein, 111 aa, synthetic construct
  source 1..111: note = Light chain variable region
QSVLTQPPSASGTPGQRVTISCTGSSSNIGSNDVTWYQQLPGTAPKLLIYADSKRPSGVPDRFSGSKSGTSASLAISGLRSEDEADYYCGTWDYSLSGYVFGGGTKLTVLG

SEQ ID NO: 57 - protein, 111 aa, synthetic construct
  source 1..111: note = Light chain variable region
QSVLTQPPSASGTPGQRVTISCSGSSSNIGSNYVSWYQQLPGTAPKLLIYDDSHRPSGVPDRFSGSKSGTSASLAISGLRSEDEADYYCGAWDDSLSGYVFGGGTKLTVLG

SEQ ID NO: 58 - protein, 111 aa, synthetic construct
  source 1..111: note = Light chain variable region
QSVLTQPPSASGTPGQRVTISCSGSSSNIGNNDVSWYQQLPGTAPKLLIYDDSQRPSGVPDRFSGSKSGTSASLAISGLRSEDEADYYCGAWDDSLSGYVFGGGTKLTVLG

SEQ ID NO: 59 - protein, 446 aa, synthetic construct
  source 1..446: note = Heavy chain
EVQLLESGGGLVQPGGSLRLSCAASGFTFSSYDMSWVRQAPGKGLEWVSWISPDSGSIYYADSVKGRFTISRDNSKNTLYLQMNSLRAEDTAVYYCARPTGRFDYWGQGTLVTVSSASTKGPSVFPLAPSSKSTSGGTAALGCLVKDYFPEPVTVSWNSGALTSGVHTFPAVLQSSGLYSLSSVVTVPSSSLGTQTYICNVNHKPSNTKVDKKVEPKSCDKTHTCPPCPAPELLGGPSVFLFPPKPKDTLMISRTPEVTCVVVDVSHEDPEVKFNWYVDGVEVHNAKTKPREEQYNSTYRVVSVLTVLHQDWLNGKEYKCKVSNKALPAPIEKTISKAKGQPREPQVYTLPPSREEMTKNQVSLTCLVKGFYPSDIAVEWESNGQPENNYKTTPPVLDSDGSFFLYSKLTVDKSRWQQGNVFSCSVMHEALHNHYTQKSLSLSPGK

SEQ ID NO: 60 - protein, 446 aa, synthetic construct
  source 1..446: note = Heavy chain
EVQLLESGGGLVQPGGSLRLSCAASGFTFSDYYMSWVRQAPGKGLEWVSSISPDGSNTYYADSVKGRFTISRDNSKNTLYLQMNSLRAEDTAVYYCAKNLRAFDYWGQGTLVTVSSASTKGPSVFPLAPSSKSTSGGTAALGCLVKDYFPEPVTVSWNSGALTSGVHTFPAVLQSSGLYSLSSVVTVPSSSLGTQTYICNVNHKPSNTKVDKKVEPKSCDKTHTCPPCPAPELLGGPSVFLFPPKPKDTLMISRTPEVTCVVVDVSHEDPEVKFNWYVDGVEVHNAKTKPREEQYNSTYRVVSVLTVLHQDWLNGKEYKCKVSNKALPAPIEKTISKAKGQPREPQVYTLPPSREEMTKNQVSLTCLVKGFYPSDIAVEWESNGQPENNYKTTPPVLDSDGSFFLYSKLTVDKSRWQQGNVFSCSVMHEALHNHYTQKSLSLSPGK

SEQ ID NO: 61 - protein, 446 aa, synthetic construct
  source 1..446: note = Heavy chain
EVQLLESGGGLVQPGGSLRLSCAASGFTFSSYDMSWVRQAPGKGLEWVSWISPGGGSKYYADSVKGRFTISRDNSKNTLYLQMNSLRAEDTAVYYCARVNGRFDYWGQGTLVTVSSASTKGPSVFPLAPSSKSTSGGTAALGCLVKDYFPEPVTVSWNSGALTSGVHTFPAVLQSSGLYSLSSVVTVPSSSLGTQTYICNVNHKPSNTKVDKKVEPKSCDKTHTCPPCPAPELLGGPSVFLFPPKPKDTLMISRTPEVTCVVVDVSHEDPEVKFNWYVDGVEVHNAKTKPREEQYNSTYRVVSVLTVLHQDWLNGKEYKCKVSNKALPAPIEKTISKAKGQPREPQVYTLPPSREEMTKNQVSLTCLVKGFYPSDIAVEWESNGQPENNYKTTPPVLDSDGSFFLYSKLTVDKSRWQQGNVFSCSVMHEALHNHYTQKSLSLSPGK

SEQ ID NO: 62 - protein, 451 aa, synthetic construct
  source 1..451: note = Heavy chain
EVQLLESGGGLVQPGGSLRLSCAASGFTFSNYDMSWVRQAPGKGLEWVSAIYHSGSSKYYADSVKGRFTISRDNSKNTLYLQMNSLRAEDTAVYYCARGGNGAWDTGFDYWGQGTLVTVSSASTKGPSVFPLAPSSKSTSGGTAALGCLVKDYFPEPVTVSWNSGALTSGVHTFPAVLQSSGLYSLSSVVTVPSSSLGTQTYICNVNHKPSNTKVDKKVEPKSCDKTHTCPPCPAPELLGGPSVFLFPPKPKDTLMISRTPEVTCVVVDVSHEDPEVKFNWYVDGVEVHNAKTKPREEQYNSTYRVVSVLTVLHQDWLNGKEYKCKVSNKALPAPIEKTISKAKGQPREPQVYTLPPSREEMTKNQVSLTCLVKGFYPSDIAVEWESNGQPENNYKTTPPVLDSDGSFFLYSKLTVDKSRWQQGNVFSCSVMHEALHNHYTQKSLSLSPGK

SEQ ID NO: 63 - protein, 457 aa, synthetic construct
  source 1..457: note = Heavy chain
EVQLLESGGGLVQPGGSLRLSCAASGFTFSSYDMSWVRQAPGKGLEWVSGISHGSGNKYYADSVKGRFTISRDNSKNTLYLQMNSLRAEDTAVYYCAKRLSLRRRPSYYSDNAMDVWGQGTLVTVSSASTKGPSVFPLAPSSKSTSGGTAALGCLVKDYFPEPVTVSWNSGALTSGVHTFPAVLQSSGLYSLSSVVTVPSSSLGTQTYICNVNHKPSNTKVDKKVEPKSCDKTHTCPPCPAPELLGGPSVFLFPPKPKDTLMISRTPEVTCVVVDVSHEDPEVKFNWYVDGVEVHNAKTKPREEQYNSTYRVVSVLTVLHQDWLNGKEYKCKVSNKALPAPIEKTISKAKGQPREPQVYTLPPSREEMTKNQVSLTCLVKGFYPSDIAVEWESNGQPENNYKTTPPVLDSDGSFFLYSKLTVDKSRWQQGNVFSCSVMHEALHNHYTQKSLSLSPGK

SEQ ID NO: 64 - protein, 457 aa, synthetic construct
  source 1..457: note = Heavy chain
EVQLLESGGGLVQPGGSLRLSCAASGFTFSNYAMSWVRQAPGKGLEWVSSISHNSGSTYYADSVKGRFTISRDNSKNTLYLQMNSLRAEDTAVYYCAKFISARKSLGRSYSNGMDVWGQGTLVTVSSASTKGPSVFPLAPSSKSTSGGTAALGCLVKDYFPEPVTVSWNSGALTSGVHTFPAVLQSSGLYSLSSVVTVPSSSLGTQTYICNVNHKPSNTKVDKKVEPKSCDKTHTCPPCPAPELLGGPSVFLFPPKPKDTLMISRTPEVTCVVVDVSHEDPEVKFNWYVDGVEVHNAKTKPREEQYNSTYRVVSVLTVLHQDWLNGKEYKCKVSNKALPAPIEKTISKAKGQPREPQVYTLPPSREEMTKNQVSLTCLVKGFYPSDIAVEWESNGQPENNYKTTPPVLDSDGSFFLYSKLTVDKSRWQQGNVFSCSVMHEALHNHYTQKSLSLSPGK

SEQ ID NO: 65 - protein, 457 aa, synthetic construct
  source 1..457: note = Heavy chain
EVQLLESGGGLVQPGGSLRLSCAASGFTFSDYDMSWVRQAPGKGLEWVSVISPDGGSIYYADSVKGRFTISRDNSKNTLYLQMNSLRAEDTAVYYCARDVVECNMNPCSYDNAMDVWGQGTLVTVSSASTKGPSVFPLAPSSKSTSGGTAALGCLVKDYFPEPVTVSWNSGALTSGVHTFPAVLQSSGLYSLSSVVTVPSSSLGTQTYICNVNHKPSNTKVDKKVEPKSCDKTHTCPPCPAPELLGGPSVFLFPPKPKDTLMISRTPEVTCVVVDVSHEDPEVKFNWYVDGVEVHNAKTKPREEQYNSTYRVVSVLTVLHQDWLNGKEYKCKVSNKALPAPIEKTISKAKGQPREPQVYTLPPSREEMTKNQVSLTCLVKGFYPSDIAVEWESNGQPENNYKTTPPVLDSDGSFFLYSKLTVDKSRWQQGNVFSCSVMHEALHNHYTQKSLSLSPGK

SEQ ID NO: 66 - protein, 458 aa, synthetic construct
  source 1..458: note = Heavy chain
EVQLLESGGGLVQPGGSLRLSCAASGFTFSNYDMSWVRQAPGKGLEWVSSISPSSGSSIYYADSVKGRFTISRDNSKNTLYLQMNSLRAEDTAVYYCAKAPGWCQAPSCYYDNAMDVWGQGTLVTVSSASTKGPSVFPLAPSSKSTSGGTAALGCLVKDYFPEPVTVSWNSGALTSGVHTFPAVLQSSGLYSLSSVVTVPSSSLGTQTYICNVNHKPSNTKVDKKVEPKSCDKTHTCPPCPAPELLGGPSVFLFPPKPKDTLMISRTPEVTCVVVDVSHEDPEVKFNWYVDGVEVHNAKTKPREEQYNSTYRVVSVLTVLHQDWLNGKEYKCKVSNKALPAPIEKTISKAKGQPREPQVYTLPPSREEMTKNQVSLTCLVKGFYPSDIAVEWESNGQPENNYKTTPPVLDSDGSFFLYSKLTVDKSRWQQGNVFSCSVMHEALHNHYTQKSLSLSPGK

SEQ ID NO: 67 - protein, 216 aa, synthetic construct
  source 1..216: note = Light chain
QSVLTQPPSASGTPGQRVTISCSGSSSNIGNNNVNWYQQLPGTAPKLLIYYDNKRPSGVPDRFSGSKSGTSASLAISGLRSEDEADYYCGTWDASLSGYVFGGGTKLTVLGQPKAAPSVTLFPPSSEELQANKATLVCLISDFYPGAVTVAWKADSSPVKAGVETTTPSKQSNNKYAASSYLSLTPEQWKSHRSYSCQVTHEGSTVEKTVAPAECS

SEQ ID NO: 68 - protein, 216 aa, synthetic construct
  source 1..216: note = Light chain
QSVLTQPPPASGTPGQRVTISCSGSSSNIGSNTVYWYQQLPGTAPKLLIYANSQRPSGVPDRFSGSKSGTSASLAISGLRSEDEADYYCGSWDYSLSGYVFGGGTKLTVLGQPKAAPSVTLFPPSSEELQANKATLVCLISDFYPGAVTVAWKADSSPVKAGVETTTPSKQSNNKYAASSYLSLTPEQWKSHRSYSCQVTHEGSTVEKTVAPAECS

SEQ ID NO: 69 - protein, 216 aa, synthetic construct
  source 1..216: note = Light chain
QSVLTQPPSASGTPGQRVTISCSGSSSNIGNNNVSWYQQLPGTAPKLLIYADSHRPSGVPDRFSGSKSGTSASLAISGLRSEDEADYYCATWDYSLSGYVFGGGTKLTVLGQPKAAPSVTLFPPSSEELQANKATLVCLISDFYPGAVTVAWKADSSPVKAGVETTTPSKQSNNKYAASSYLSLTPEQWKSHRSYSCQVTHEGSTVEKTVAPAECS

SEQ ID NO: 70 - protein, 216 aa, synthetic construct
  source 1..216: note = Light chain
QSVLTQPPSASGTPGQRVTISCSGSSSNIGSNDVSWYQQLPGTAPKLLIYYDNNRPSGVPDRFSGSKSGTSASLAISGLRSEDEADYYCGAWDDSLSGYVFGGGTKLTVLGQPKAAPSVTLFPPSSEELQANKATLVCLISDFYPGAVTVAWKADSSPVKAGVETTTPSKQSNNKYAASSYLSLTPEQWKSHRSYSCQVTHEGSTVEKTVAPAECS

SEQ ID NO: 71 - protein, 216 aa, synthetic construct
  source 1..216: note = Light chain
QSVLTQPPSASGTPGQRVTISCTGSSSNIGNNAVNWYQQLPGTAPKLLIYYDSNRPSGVPDRFSGSKSGTSASLAISGLRSEDEADYYCGAWDDSLSGYVFGGGTKLTVLGQPKAAPSVTLFPPSSEELQANKATLVCLISDFYPGAVTVAWKADSSPVKAGVETTTPSKQSNNKYAASSYLSLTPEQWKSHRSYSCQVTHEGSTVEKTVAPAECS

SEQ ID NO: 72 - protein, 216 aa, synthetic construct
  source 1..216: note = Light chain
QSVLTQPPSASGTPGQRVTISCTGSSSNIGSNDVTWYQQLPGTAPKLLIYADSKRPSGVPDRFSGSKSGTSASLAISGLRSEDEADYYCGTWDYSLSGYVFGGGTKLTVLGQPKAAPSVTLFPPSSEELQANKATLVCLISDFYPGAVTVAWKADSSPVKAGVETTTPSKQSNNKYAASSYLSLTPEQWKSHRSYSCQVTHEGSTVEKTVAPAECS

SEQ ID NO: 73 - protein, 216 aa, synthetic construct
  source 1..216: note = Light chain
QSVLTQPPSASGTPGQRVTISCSGSSSNIGSNYVSWYQQLPGTAPKLLIYDDSHRPSGVPDRFSGSKSGTSASLAISGLRSEDEADYYCGAWDDSLSGYVFGGGTKLTVLGQPKAAPSVTLFPPSSEELQANKATLVCLISDFYPGAVTVAWKADSSPVKAGVETTTPSKQSNNKYAASSYLSLTPEQWKSHRSYSCQVTHEGSTVEKTVAPAECS

SEQ ID NO: 74 - protein, 216 aa, synthetic construct
  source 1..216: note = Light chain
QSVLTQPPSASGTPGQRVTISCSGSSSNIGNNDVSWYQQLPGTAPKLLIYDDSQRPSGVPDRFSGSKSGTSASLAISGLRSEDEADYYCGAWDDSLSGYVFGGGTKLTVLGQPKAAPSVTLFPPSSEELQANKATLVCLISDFYPGAVTVAWKADSSPVKAGVETTTPSKQSNNKYAASSYLSLTPEQWKSHRSYSCQVTHEGSTVEKTVAPAECS

SEQ ID NO: 75 - DNA, 1338 bp, synthetic construct
  source 1..1338: mol_type = other DNA; note = Heavy chain coding gene
gaagtacaacttctggagtcaggtggaggacttgttcagcccggcgggtccctgaggctgagttgcgcagcaagcgggttcacattctcctcttatgatatgtcttgggtaagacaggctcctggtaagggtctggaatgggtatcctggataagtcctgactccggttcaatatactacgccgatagtgtgaagggacgtttcaccatcagccgggacaacagcaaaaataccttgtatctccaaatgaatagcctccgggctgaagacactgccgtatattactgcgccagacctactggtcgttttgactattgggggcaaggaacactggtaaccgtttcaagcgcctccaccaagggcccctccgtgttccccctggccccctcctccaagtccacctccggcggcaccgccgccctgggctgcctggtgaaggactacttccccgagcccgtgaccgtgtcctggaactccggcgccctgacctccggcgtgcacaccttccccgccgtgctgcagtcctccggcctgtactccctgtcctccgtcgtgaccgtgccctcctcctccctgggcacccagacctacatctgcaacgtgaaccacaagccctccaacaccaaggtggacaagaaggtggagcccaagtcctgcgacaagacccacacctgccctccctgccccgcccccgagctgctgggcggcccctccgtgttcctgttccctcctaagcccaaggacaccctgatgatctcccggacccccgaggtgacttgcgtggtggtggacgtgtcccacgaggaccccgaggtgaagttcaactggtacgtggacggcgtggaggtgcacaacgccaagaccaagccccgggaggagcagtacaactccacctaccgggtggtgtccgtgctgaccgtgctgcaccaggactggctgaacggcaaggagtacaagtgcaaggtgtccaacaaggccctgcccgcccccatcgagaagaccatctccaaggccaagggccagccccgggagccccaggtgtacaccctgcccccctcccgggaggagatgaccaagaaccaggtgtccctgacctgcctggtgaagggcttctacccctccgacatcgccgtggagtgggagtccaacggccagcccgagaacaactacaagaccaccccccccgtgctggactccgacggctccttcttcctgtactccaagctgaccgtggacaagtcccggtggcagcagggcaacgtgttctcctgctccgtgatgcacgaggccctgcacaaccactacacccagaagtccctgtccctgtcccccggcaag

SEQ ID NO: 76 - DNA, 1338 bp, synthetic construct
  source 1..1338: mol_type = other DNA; note = Heavy chain coding gene
gaagtgcagctgctggaatccggcggaggcctggtgcagcctggcggctctctgagactgtcttgcgccgcctccggcttcaccttctccgactactacatgtcctgggtgcgacaggcccctggcaagggcctggaatgggtgtcctccatctcccccgacggctccaacacctactacgccgactccgtgaagggccggttcaccatctcccgggacaactccaagaacaccctgtacctgcagatgaactccctgcgggccgaggacaccgccgtgtactactgcgccaagaacctgcgggccttcgactactggggccagggcacactggtgaccgtgtcctccgcctccaccaagggcccctccgtgttccccctggccccctcctccaagtccacctccggcggcaccgccgccctgggctgcctggtgaaggactacttccccgagcccgtgaccgtgtcctggaactccggcgccctgacctccggcgtgcacaccttccccgccgtgctgcagtcctccggcctgtactccctgtcctccgtcgtgaccgtgccctcctcctccctgggcacccagacctacatctgcaacgtgaaccacaagccctccaacaccaaggtggacaagaaggtggagcccaagtcctgcgacaagacccacacctgccctccctgccccgcccccgagctgctgggcggcccctccgtgttcctgttccctcctaagcccaaggacaccctgatgatctcccggacccccgaggtgacttgcgtggtggtggacgtgtcccacgaggaccccgaggtgaagttcaactggtacgtggacggcgtggaggtgcacaacgccaagaccaagccccgggaggagcagtacaactccacctaccgggtggtgtccgtgctgaccgtgctgcaccaggactggctgaacggcaaggagtacaagtgcaaggtgtccaacaaggccctgcccgcccccatcgagaagaccatctccaaggccaagggccagccccgggagccccaggtgtacaccctgcccccctcccgggaggagatgaccaagaaccaggtgtccctgacctgcctggtgaagggcttctacccctccgacatcgccgtggagtgggagtccaacggccagcccgagaacaactacaagaccaccccccccgtgctggactccgacggctccttcttcctgtactccaagctgaccgtggacaagtcccggtggcagcagggcaacgtgttctcctgctccgtgatgcacgaggccctgcacaaccactacacccagaagtccctgtccctgtcccccggcaag

SEQ ID NO: 77 - DNA, 1341 bp, synthetic construct
  source 1..1341: mol_type = other DNA; note = Heavy chain coding gene
gaagtgcaacttcttgagagtggtggaggattggtacaacctgggggtagtttgcgtctctcctgtgctgcttctggtttcacattttcctcctatgacatgagctgggtacggcaagctccaggaaaagggcttgagtgggtctcctggatctctcccggtggaggcagcaagtattatgcagactctgtaaagggtaggtttactatatcacgcgataatagtaagaatactttgtatttgcaaatgaactccctccgagctgaggacacagcagtctattattgcgcccgagttaacggtcgcttcgattactggggccaaggcacactggttacagtgtcctcagcctccaccaagggcccctccgtgttccccctggccccctcctccaagtccacctccggcggcaccgccgccctgggctgcctggtgaaggactacttccccgagcccgtgaccgtgtcctggaactccggcgccctgacctccggcgtgcacaccttccccgccgtgctgcagtcctccggcctgtactccctgtcctccgtcgtgaccgtgccctcctcctccctgggcacccagacctacatctgcaacgtgaaccacaagccctccaacaccaaggtggacaagaaggtggagcccaagtcctgcgacaagacccacacctgccctccctgccccgcccccgagctgctgggcggcccctccgtgttcctgttccctcctaagcccaaggacaccctgatgatctcccggacccccgaggtgacttgcgtggtggtggacgtgtcccacgaggaccccgaggtgaagttcaactggtacgtggacggcgtggaggtgcacaacgccaagaccaagccccgggaggagcagtacaactccacctaccgggtggtgtccgtgctgaccgtgctgcaccaggactggctgaacggcaaggagtacaagtgcaaggtgtccaacaaggccctgcccgcccccatcgagaagaccatctccaaggccaagggccagccccgggagccccaggtgtacaccctgcccccctcccgggaggagatgaccaagaaccaggtgtccctgacctgcctggtgaagggcttctacccctccgacatcgccgtggagtgggagtccaacggccagcccgagaacaactacaagaccaccccccccgtgctggactccgacggctccttcttcctgtactccaagctgaccgtggacaagtcccggtggcagcagggcaacgtgttctcctgctccgtgatgcacgaggccctgcacaaccactacacccagaagtccctgtccctgtcccccggcaagtga

SEQ ID NO: 78 - DNA, 1353 bp, synthetic construct
  source 1..1353: mol_type = other DNA; note = Heavy chain coding gene
gaggtgcagctgctggagtccggcggcggcctggtgcagcccggcggctccctgcggctgtcctgcgccgcctccggcttcaccttctccaactacgacatgtcctgggtgcggcaggcccccggcaagggcctggagtgggtgtccgccatctaccactccggctcctccaagtactacgccgactccgtgaagggccggttcaccatctcccgggacaactccaagaacaccctgtacctgcagatgaactccctgcgggccgaggacaccgccgtgtactactgcgcccggggcggcaacggcgcctgggacaccggcttcgactactggggccagggcaccctggtgaccgtgtcctccgcctccaccaagggcccctccgtgttccccctggccccctcctccaagtccacctccggcggcaccgccgccctgggctgcctggtgaaggactacttccccgagcccgtgaccgtgtcctggaactccggcgccctgacctccggcgtgcacaccttccccgccgtgctgcagtcctccggcctgtactccctgtcctccgtcgtgaccgtgccctcctcctccctgggcacccagacctacatctgcaacgtgaaccacaagccctccaacaccaaggtggacaagaaggtggagcccaagtcctgcgacaagacccacacctgccctccctgccccgcccccgagctgctgggcggcccctccgtgttcctgttccctcctaagcccaaggacaccctgatgatctcccggacccccgaggtgacttgcgtggtggtggacgtgtcccacgaggaccccgaggtgaagttcaactggtacgtggacggcgtggaggtgcacaacgccaagaccaagccccgggaggagcagtacaactccacctaccgggtggtgtccgtgctgaccgtgctgcaccaggactggctgaacggcaaggagtacaagtgcaaggtgtccaacaaggccctgcccgcccccatcgagaagaccatctccaaggccaagggccagccccgggagccccaggtgtacaccctgcccccctcccgggaggagatgaccaagaaccaggtgtccctgacctgcctggtgaagggcttctacccctccgacatcgccgtggagtgggagtccaacggccagcccgagaacaactacaagaccaccccccccgtgctggactccgacggctccttcttcctgtactccaagctgaccgtggacaagtcccggtggcagcagggcaacgtgttctcctgctccgtgatgcacgaggccctgcacaaccactacacccagaagtccctgtccctgtcccccggcaag

SEQ ID NO: 79 - DNA, 1374 bp, synthetic construct
  source 1..1374: mol_type = other DNA; note = Heavy chain coding gene
gaagttcaactgttggaatccgggggtggtctggtccaacctggagggtctcttagactgagttgtgctgcttcaggcttcacatttagctcatatgatatgtcctgggtcagacaggcccccggcaaaggtcttgaatgggtatctggtattagtcatggatctggcaacaagtactacgctgatagtgtcaaaggacgattcaccatatctcgtgacaactctaaaaacactttgtacttgcagatgaactcactgcgtgccgaagacacagccgtgtattattgcgctaagcgtctctcactccgcaggcgaccttcctattacagcgacaacgctatggatgtctgggggcagggtacactcgtcaccgtgtcatcagcctccaccaagggcccctccgtgttccccctggccccctcctccaagtccacctccggcggcaccgccgccctgggctgcctggtgaaggactacttccccgagcccgtgaccgtgtcctggaactccggcgccctgacctccggcgtgcacaccttccccgccgtgctgcagtcctccggcctgtactccctgtcctccgtcgtgaccgtgccctcctcctccctgggcacccagacctacatctgcaacgtgaaccacaagccctccaacaccaaggtggacaagaaggtggagcccaagtcctgcgacaagacccacacctgccctccctgccccgcccccgagctgctgggcggcccctccgtgttcctgttccctcctaagcccaaggacaccctgatgatctcccggacccccgaggtgacttgcgtggtggtggacgtgtcccacgaggaccccgaggtgaagttcaactggtacgtggacggcgtggaggtgcacaacgccaagaccaagccccgggaggagcagtacaactccacctaccgggtggtgtccgtgctgaccgtgctgcaccaggactggctgaacggcaaggagtacaagtgcaaggtgtccaacaaggccctgcccgcccccatcgagaagaccatctccaaggccaagggccagccccgggagccccaggtgtacaccctgcccccctcccgggaggagatgaccaagaaccaggtgtccctgacctgcctggtgaagggcttctacccctccgacatcgccgtggagtgggagtccaacggccagcccgagaacaactacaagaccaccccccccgtgctggactccgacggctccttcttcctgtactccaagctgaccgtggacaagtcccggtggcagcagggcaacgtgttctcctgctccgtgatgcacgaggccctgcacaaccactacacccagaagtccctgtccctgtcccccggcaagtga

SEQ ID NO: 80 - DNA, 1371 bp, synthetic construct
  source 1..1371: mol_type = other DNA; note = Heavy chain coding gene
gaggtgcagctgctggagtccggcggcggcctggtgcagcccggcggctccctgcggctgtcctgcgccgcctccggcttcaccttctccaactacgccatgtcctgggtgcggcaggcccccggcaagggcctggagtgggtgtcctccatctcccacaactccggctccacctactacgccgactccgtgaagggccggttcaccatctcccgggacaactccaagaacaccctgtacctgcagatgaactccctgcgggccgaggacaccgccgtgtactactgcgccaagttcatctccgcccggaagtccctgggccggtcctactccaacggcatggacgtgtggggccagggcaccctggtgaccgtgtcctccgcctccaccaagggcccctccgtgttccccctggccccctcctccaagtccacctccggcggcaccgccgccctgggctgcctggtgaaggactacttccccgagcccgtgaccgtgtcctggaactccggcgccctgacctccggcgtgcacaccttccccgccgtgctgcagtcctccggcctgtactccctgtcctccgtcgtgaccgtgccctcctcctccctgggcacccagacctacatctgcaacgtgaaccacaagccctccaacaccaaggtggacaagaaggtggagcccaagtcctgcgacaagacccacacctgccctccctgccccgcccccgagctgctgggcggcccctccgtgttcctgttccctcctaagcccaaggacaccctgatgatctcccggacccccgaggtgacttgcgtggtggtggacgtgtcccacgaggaccccgaggtgaagttcaactggtacgtggacggcgtggaggtgcacaacgccaagaccaagccccgggaggagcagtacaactccacctaccgggtggtgtccgtgctgaccgtgctgcaccaggactggctgaacggcaaggagtacaagtgcaaggtgtccaacaaggccctgcccgcccccatcgagaagaccatctccaaggccaagggccagccccgggagccccaggtgtacaccctgcccccctcccgggaggagatgaccaagaaccaggtgtccctgacctgcctggtgaagggcttctacccctccgacatcgccgtggagtgggagtccaacggccagcccgagaacaactacaagaccaccccccccgtgctggactccgacggctccttcttcctgtactccaagctgaccgtggacaagtcccggtggcagcagggcaacgtgttctcctgctccgtgatgcacgaggccctgcacaaccactacacccagaagtccctgtccctgtcccccggcaag

SEQ ID NO: 81 - DNA, 1371 bp, synthetic construct
  source 1..1371: mol_type = other DNA; note = Heavy chain coding gene
gaagtacagttgcttgaaagtggcggtggtcttgtccagccaggcggttcccttcggctgtcttgcgccgcaagtggcttcactttcagcgactatgatatgtcttgggtccgccaagcaccaggaaagggacttgaatgggtgagtgtaatcagtcctgacggagggtcaatttattatgcagattcagtcaagggtcgattcactatatcccgagacaactccaaaaatactctttatcttcagatgaactctttgagagctgaagacaccgcagtttattactgtgctcgggatgtagtggagtgcaatatgaatccctgctcatacgacaacgcaatggatgtttgggggcaggggactctggtgacagtcagctctgcctccaccaagggcccctccgtgttccccctggccccctcctccaagtccacctccggcggcaccgccgccctgggctgcctggtgaaggactacttccccgagcccgtgaccgtgtcctggaactccggcgccctgacctccggcgtgcacaccttccccgccgtgctgcagtcctccggcctgtactccctgtcctccgtcgtgaccgtgccctcctcctccctgggcacccagacctacatctgcaacgtgaaccacaagccctccaacaccaaggtggacaagaaggtggagcccaagtcctgcgacaagacccacacctgccctccctgccccgcccccgagctgctgggcggcccctccgtgttcctgttccctcctaagcccaaggacaccctgatgatctcccggacccccgaggtgacttgcgtggtggtggacgtgtcccacgaggaccccgaggtgaagttcaactggtacgtggacggcgtggaggtgcacaacgccaagaccaagccccgggaggagcagtacaactccacctaccgggtggtgtccgtgctgaccgtgctgcaccaggactggctgaacggcaaggagtacaagtgcaaggtgtccaacaaggccctgcccgcccccatcgagaagaccatctccaaggccaagggccagccccgggagccccaggtgtacaccctgcccccctcccgggaggagatgaccaagaaccaggtgtccctgacctgcctggtgaagggcttctacccctccgacatcgccgtggagtgggagtccaacggccagcccgagaacaactacaagaccaccccccccgtgctggactccgacggctccttcttcctgtactccaagctgaccgtggacaagtcccggtggcagcagggcaacgtgttctcctgctccgtgatgcacgaggccctgcacaaccactacacccagaagtccctgtccctgtcccccggcaag

SEQ ID NO: 82 - DNA, 1374 bp, synthetic construct
  source 1..1374: mol_type = other DNA; note = Heavy chain coding gene
gaagtgcagctgcttgaatcaggaggcggcctcgtacaaccagggggatctctcagactgtcctgcgctgccagtggcttcactttcagcaactacgatatgtcatgggtgaggcaggcacctggcaagggtctggagtgggtctcaagcataagtcccagtagtggaagctcaatttattacgccgacagtgtaaagggccggttcaccattagtagagacaattctaagaataccttgtaccttcaaatgaatagtctgagagccgaagataccgcagtttattattgcgctaaggccccagggtggtgtcaggccccttcatgctattatgataatgcaatggacgtgtggggtcagggtactctggtcacagtcagtagtgcctccaccaagggcccctccgtgttccccctggccccctcctccaagtccacctccggcggcaccgccgccctgggctgcctggtgaaggactacttccccgagcccgtgaccgtgtcctggaactccggcgccctgacctccggcgtgcacaccttccccgccgtgctgcagtcctccggcctgtactccctgtcctccgtcgtgaccgtgccctcctcctccctgggcacccagacctacatctgcaacgtgaaccacaagccctccaacaccaaggtggacaagaaggtggagcccaagtcctgcgacaagacccacacctgccctccctgccccgcccccgagctgctgggcggcccctccgtgttcctgttccctcctaagcccaaggacaccctgatgatctcccggacccccgaggtgacttgcgtggtggtggacgtgtcccacgaggaccccgaggtgaagttcaactggtacgtggacggcgtggaggtgcacaacgccaagaccaagccccgggaggagcagtacaactccacctaccgggtggtgtccgtgctgaccgtgctgcaccaggactggctgaacggcaaggagtacaagtgcaaggtgtccaacaaggccctgcccgcccccatcgagaagaccatctccaaggccaagggccagccccgggagccccaggtgtacaccctgcccccctcccgggaggagatgaccaagaaccaggtgtccctgacctgcctggtgaagggcttctacccctccgacatcgccgtggagtgggagtccaacggccagcccgagaacaactacaagaccaccccccccgtgctggactccgacggctccttcttcctgtactccaagctgaccgtggacaagtcccggtggcagcagggcaacgtgttctcctgctccgtgatgcacgaggccctgcacaaccactacacccagaagtccctgtccctgtcccccggcaag

SEQ ID NO: 83 - DNA, 648 bp, synthetic construct
  source 1..648: mol_type = other DNA; note = Light chain coding gene
cagtctgtgctgacacaaccaccttctgcctctgggactccaggccagcgggttaccattagctgttctggtagttctagtaatatcggtaacaacaatgtgaattggtatcaacaactgccaggaaccgcccctaagttgctcatatattatgataacaagcggccttcaggcgttcctgatcgtttctccggctctaaaagtggcacatccgccagtcttgctatcagcggtctcagatccgaggacgaggccgactattattgtggtacatgggacgcttccctgtcaggttacgtctttggcggcggcacaaaactgacagttcttggccagcccaaggccgccccctccgtgaccctgttccccccctcctccgaggagctgcaggccaacaaggccaccctggtgtgcctgatctccgacttctaccccggcgccgtgaccgtggcctggaaggccgactcctcccccgtgaaggccggcgtggagaccaccaccccctccaagcagtccaacaacaagtacgccgcctcctcctacctgtccctgacccccgagcagtggaagtcccaccggtcctactcctgccaggtgacccacgagggctccaccgtggagaagaccgtggcccccgccgagtgctcc

SEQ ID NO: 84 - DNA, 648 bp, synthetic construct
  source 1..648: mol_type = other DNA; note = Light chain coding gene
cagtctgtgctgacccagcctccccctgcttctggcacccctggccagagagtgaccatctcctgctccggctcctcctccaacatcggctccaacaccgtgtactggtatcagcagctgcccggcaccgcccccaagctgctgatctacgccaactcccagcggccctccggcgtgcccgacagattctccggctccaagtccggcacctccgcctccctggccatctccggcctgagatctgaggacgaggccgactactactgcggctcctgggactactccctgtccggctacgtgttcggcggaggcaccaagctgaccgtgctgggccagcctaaggccgctccctccgtgaccctgttccccccatcctccgaggaactgcaggccaacaaggccaccctggtctgcctgatctccgacttctaccctggcgccgtgaccgtggcctggaaggccgacagctctcctgtgaaggccggcgtggaaaccaccaccccctccaagcagtccaacaacaaatacgccgcctcctcctacctgtccctgacccccgagcagtggaagtcccaccggtcctacagctgccaggtcacacacgagggctccaccgtggaaaagaccgtggcccctgccgagtgctcc

SEQ ID NO: 85 - DNA, 648 bp, synthetic construct
  source 1..648: mol_type = other DNA; note = Light chain coding gene
cagagtgttttgacccagcctccttccgccagcggcacccctgggcaacgggttacaatcagctgttccgggagcagcagtaacattggtaataataacgtctcttggtatcagcagttgcctggcacagcacctaagctcctgatttacgctgactcccaccggccttccggcgtccctgatcgtttctccgggtcaaaaagtggaacctcagcaagccttgcaatcagcggactgcggtccgaagatgaagctgactactactgcgctacctgggattactcattgtccggctacgtctttggggggggaaccaaattgacagtcttgggtcagcccaaggccgccccctccgtgaccctgttccccccctcctccgaggagctgcaggccaacaaggccaccctggtgtgcctgatctccgacttctaccccggcgccgtgaccgtggcctggaaggccgactcctcccccgtgaaggccggcgtggagaccaccaccccctccaagcagtccaacaacaagtacgccgcctcctcctacctgtccctgacccccgagcagtggaagtcccaccggtcctactcctgccaggtgacccacgagggctccaccgtggagaagaccgtggcccccgccgagtgctcc

SEQ ID NO: 86 - DNA, 648 bp, synthetic construct
  source 1..648: mol_type = other DNA; note = Light chain coding gene
cagtccgtgctgacccagcccccctccgcctccggcacccccggccagcgggtgaccatctcctgctccggctcctcctccaacatcggctccaacgacgtgtcctggtaccagcagctgcccggcaccgcccccaagctgctgatctactacgacaacaaccggccctccggcgtgcccgaccggttctccggctccaagtccggcacctccgcctccctggccatctccggcctgcggtccgaggacgaggccgactactactgcggcgcctgggacgactccctgtccggctacgtgttcggcggcggcaccaagctgaccgtgctgggccagcccaaggccgccccctccgtgaccctgttccccccctcctccgaggagctgcaggccaacaaggccaccctggtgtgcctgatctccgacttctaccccggcgccgtgaccgtggcctggaaggccgactcctcccccgtgaaggccggcgtggagaccaccaccccctccaagcagtccaacaacaagtacgccgcctcctcctacctgtccctgacccccgagcagtggaagtcccaccggtcctactcctgccaggtgacccacgagggctccaccgtggagaagaccgtggcccccgccgagtgctcc

SEQ ID NO: 87 - DNA, 651 bp, synthetic construct
  source 1..651: mol_type = other DNA; note = Light chain coding gene
caaagcgtactcacccagcccccatccgcatctggcactcctggtcaacgggttacaatctcttgtactgggtcaagttccaatattggaaataacgcagtgaactggtatcagcagctccctggcaccgcccctaaactcttgatatactatgactctaatcggccaagtggagtccccgataggttctcaggttctaagagtggcacaagtgccagcctggcaatctcagggctcaggtccgaagatgaggctgattattactgcggagcttgggatgatagcctgagtggctacgtcttcgggggaggaacaaaattgaccgtacttggccagcccaaggccgccccctccgtgaccctgttccccccctcctccgaggagctgcaggccaacaaggccaccctggtgtgcctgatctccgacttctaccccggcgccgtgaccgtggcctggaaggccgactcctcccccgtgaaggccggcgtggagaccaccaccccctccaagcagtccaacaacaagtacgccgcctcctcctacctgtccctgacccccgagcagtggaagtcccaccggtcctactcctgccaggtgacccacgagggctccaccgtggagaagaccgtggcccccgccgagtgctcctga

SEQ ID NO: 88 - DNA, 648 bp, synthetic construct
  source 1..648: mol_type = other DNA; note = Light chain coding gene
cagtccgtgctgacccagcccccctccgcctccggcacccccggccagcgggtgaccatctcctgcaccggctcctcctccaacatcggctccaacgacgtgacctggtaccagcagctgcccggcaccgcccccaagctgctgatctacgccgactccaagcggccctccggcgtgcccgaccggttctccggctccaagtccggcacctccgcctccctggccatctccggcctgcggtccgaggacgaggccgactactactgcggcacctgggactactccctgtccggctacgtgttcggcggcggcaccaagctgaccgtgctgggccagcccaaggccgccccctccgtgaccctgttccccccctcctccgaggagctgcaggccaacaaggccaccctggtgtgcctgatctccgacttctaccccggcgccgtgaccgtggcctggaaggccgactcctcccccgtgaaggccggcgtggagaccaccaccccctccaagcagtccaacaacaagtacgccgcctcctcctacctgtccctgacccccgagcagtggaagtcccaccggtcctactcctgccaggtgacccacgagggctccaccgtggagaagaccgtggcccccgccgagtgctcc

SEQ ID NO: 89 - DNA, 648 bp, synthetic construct
  source 1..648: mol_type = other DNA; note = Light chain coding gene
caaagtgtattgactcaacctccctccgcttccggtacaccagggcagcgagtaaccatcagttgcagtggcagcagctccaatatcggaagcaattatgtaagttggtatcaacagttgccagggaccgctccaaaactgttgatctatgacgacagtcaccgtccttcaggtgtgcccgaccgattttcaggcagcaagagcggcacatccgcctccctcgctatctccggcctccgatccgaagatgaggccgactactattgtggagcctgggacgactcccttagtggctatgtgtttgggggagggacaaagttgaccgtacttggccagcccaaggccgccccctccgtgaccctgttccccccctcctccgaggagctgcaggccaacaaggccaccctggtgtgcctgatctccgacttctaccccggcgccgtgaccgtggcctggaaggccgactcctcccccgtgaaggccggcgtggagaccaccaccccctccaagcagtccaacaacaagtacgccgcctcctcctacctgtccctgacccccgagcagtggaagtcccaccggtcctactcctgccaggtgacccacgagggctccaccgtggagaagaccgtggcccccgccgagtgctcc

SEQ ID NO: 90 - DNA, 648 bp, synthetic construct
  source 1..648: mol_type = other DNA; note = Light chain coding gene
cagtcagttcttacacaacccccatccgcttctggcactcccggccagcgcgtaactatatcttgctctgggagtagtagcaatatcggtaataatgatgtctcatggtaccaacagctgcctggaacagcccccaaactcctcatttatgatgactctcaaaggccaagtggtgtgccagacagattttccggtagcaagagtggaacatcagcaagtcttgctataagtggcttgcgttccgaggacgaggccgactattattgtggcgcatgggatgactcactgagcggctacgttttcgggggcggtactaagttgaccgttttgggacagcccaaggccgccccctccgtgaccctgttccccccctcctccgaggagctgcaggccaacaaggccaccctggtgtgcctgatctccgacttctaccccggcgccgtgaccgtggcctggaaggccgactcctcccccgtgaaggccggcgtggagaccaccaccccctccaagcagtccaacaacaagtacgccgcctcctcctacctgtccctgacccccgagcagtggaagtcccaccggtcctactcctgccaggtgacccacgagggctccaccgtggagaagaccgtggcccccgccgagtgctcc

SEQ ID NO: 91 - protein, 330 aa, synthetic construct
  source 1..330: note = Heavy chain constant region
ASTKGPSVFPLAPSSKSTSGGTAALGCLVKDYFPEPVTVSWNSGALTSGVHTFPAVLQSSGLYSLSSVVTVPSSSLGTQTYICNVNHKPSNTKVDKKVEPKSCDKTHTCPPCPAPELLGGPSVFLFPPKPKDTLMISRTPEVTCVVVDVSHEDPEVKFNWYVDGVEVHNAKTKPREEQYNSTYRVVSVLTVLHQDWLNGKEYKCKVSNKALPAPIEKTISKAKGQPREPQVYTLPPSREEMTKNQVSLTCLVKGFYPSDIAVEWESNGQPENNYKTTPPVLDSDGSFFLYSKLTVDKSRWQQGNVFSCSVMHEALHNHYTQKSLSLSPGK

SEQ ID NO: 92 - DNA, 993 bp, synthetic construct
  source 1..993: mol_type = other DNA; note = Heavy chain constant region coding gene
gcctccaccaagggcccctccgtgttccccctggccccctcctccaagtccacctccggcggcaccgccgccctgggctgcctggtgaaggactacttccccgagcccgtgaccgtgtcctggaactccggcgccctgacctccggcgtgcacaccttccccgccgtgctgcagtcctccggcctgtactccctgtcctccgtcgtgaccgtgccctcctcctccctgggcacccagacctacatctgcaacgtgaaccacaagccctccaacaccaaggtggacaagaaggtggagcccaagtcctgcgacaagacccacacctgccctccctgccccgcccccgagctgctgggcggcccctccgtgttcctgttccctcctaagcccaaggacaccctgatgatctcccggacccccgaggtgacttgcgtggtggtggacgtgtcccacgaggaccccgaggtgaagttcaactggtacgtggacggcgtggaggtgcacaacgccaagaccaagccccgggaggagcagtacaactccacctaccgggtggtgtccgtgctgaccgtgctgcaccaggactggctgaacggcaaggagtacaagtgcaaggtgtccaacaaggccctgcccgcccccatcgagaagaccatctccaaggccaagggccagccccgggagccccaggtgtacaccctgcccccctcccgggaggagatgaccaagaaccaggtgtccctgacctgcctggtgaagggcttctacccctccgacatcgccgtggagtgggagtccaacggccagcccgagaacaactacaagaccaccccccccgtgctggactccgacggctccttcttcctgtactccaagctgaccgtggacaagtcccggtggcagcagggcaacgtgttctcctgctccgtgatgcacgaggccctgcacaaccactacacccagaagtccctgtccctgtcccccggcaagtga

SEQ ID NO: 93 - protein, 105 aa, synthetic construct
  source 1..105: note = Light chain constant region
QPKAAPSVTLFPPSSEELQANKATLVCLISDFYPGAVTVAWKADSSPVKAGVETTTPSKQSNNKYAASSYLSLTPEQWKSHRSYSCQVTHEGSTVEKTVAPAECS

SEQ ID NO: 94 - DNA, 318 bp, synthetic construct
  source 1..318: mol_type = other DNA; note = Light chain constant region coding gene
cagcccaaggccgccccctccgtgaccctgttccccccctcctccgaggagctgcaggccaacaaggccaccctggtgtgcctgatctccgacttctaccccggcgccgtgaccgtggcctggaaggccgactcctcccccgtgaaggccggcgtggagaccaccaccccctccaagcagtccaacaacaagtacgccgcctcctcctacctgtccctgacccccgagcagtggaagtcccaccggtcctactcctgccaggtgacccacgagggctccaccgtggagaagaccgtggcccccgccgagtgctcctga

SEQ ID NO: 95 - DNA, 318 bp, synthetic construct
  source 1..318: mol_type = other DNA; note = Light chain constant region coding gene
cagcctaaggccgctccctccgtgaccctgttccccccatcctccgaggaactgcaggccaacaaggccaccctggtctgcctgatctccgacttctaccctggcgccgtgaccgtggcctggaaggccgacagctctcctgtgaaggccggcgtggaaaccaccaccccctccaagcagtccaacaacaaatacgccgcctcctcctacctgtccctgacccccgagcagtggaagtcccaccggtcctacagctgccaggtcacacacgagggctccaccgtggaaaagaccgtggcccctgccgagtgctcctga

SEQ ID NO: 96 - protein, 17 aa, synthetic construct
  source 1..17: note = Heavy chain CDR2
SISPDASNTYYADSVKG

SEQ ID NO: 97 - protein, 12 aa, synthetic construct
  source 1..12: note = Heavy chain CDR3
GGNAAWDTGFDY

SEQ ID NO: 98 - protein, 116 aa, synthetic construct
  source 1..116: note = Heavy chain variable region
EVQLLESGGGLVQPGGSLRLSCAASGFTFSDYYMSWVRQAPGKGLEWVSSISPDASNTYYADSVKGRFTISRDNSKNTLYLQMNSLRAEDTAVYYCAKNLRAFDYWGQGTLVTVSS

SEQ ID NO: 99 - protein, 121 aa, synthetic construct
  source 1..121: note = Heavy chain variable region
EVQLLESGGGLVQPGGSLRLSCAASGFTFSNYDMSWVRQAPGKGLEWVSAIYHSGSSKYYADSVKGRFTISRDNSKNTLYLQMNSLRAEDTAVYYCARGGNAAWDTGFDYWGQGTLVTVSS

SEQ ID NO: 100 - protein, 446 aa, synthetic construct
  source 1..446: note = Heavy chain
EVQLLESGGGLVQPGGSLRLSCAASGFTFSDYYMSWVRQAPGKGLEWVSSISPDASNTYYADSVKGRFTISRDNSKNTLYLQMNSLRAEDTAVYYCAKNLRAFDYWGQGTLVTVSSASTKGPSVFPLAPSSKSTSGGTAALGCLVKDYFPEPVTVSWNSGALTSGVHTFPAVLQSSGLYSLSSVVTVPSSSLGTQTYICNVNHKPSNTKVDKKVEPKSCDKTHTCPPCPAPELLGGPSVFLFPPKPKDTLMISRTPEVTCVVVDVSHEDPEVKFNWYVDGVEVHNAKTKPREEQYNSTYRVVSVLTVLHQDWLNGKEYKCKVSNKALPAPIEKTISKAKGQPREPQVYTLPPSREEMTKNQVSLTCLVKGFYPSDIAVEWESNGQPENNYKTTPPVLDSDGSFFLYSKLTVDKSRWQQGNVFSCSVMHEALHNHYTQKSLSLSPGK

SEQ ID NO: 101 - protein, 451 aa, synthetic construct
  source 1..451: note = Heavy chain
EVQLLESGGGLVQPGGSLRLSCAASGFTFSNYDMSWVRQAPGKGLEWVSAIYHSGSSKYYADSVKGRFTISRDNSKNTLYLQMNSLRAEDTAVYYCARGGNAAWDTGFDYWGQGTLVTVSSASTKGPSVFPLAPSSKSTSGGTAALGCLVKDYFPEPVTVSWNSGALTSGVHTFPAVLQSSGLYSLSSVVTVPSSSLGTQTYICNVNHKPSNTKVDKKVEPKSCDKTHTCPPCPAPELLGGPSVFLFPPKPKDTLMISRTPEVTCVVVDVSHEDPEVKFNWYVDGVEVHNAKTKPREEQYNSTYRVVSVLTVLHQDWLNGKEYKCKVSNKALPAPIEKTISKAKGQPREPQVYTLPPSREEMTKNQVSLTCLVKGFYPSDIAVEWESNGQPENNYKTTPPVLDSDGSFFLYSKLTVDKSRWQQGNVFSCSVMHEALHNHYTQKSLSLSPGK

SEQ ID NO: 102 - DNA, 1338 bp, synthetic construct
  source 1..1338: mol_type = other DNA; note = Heavy chain coding gene
gaagtgcagctgctggaatccggcggaggcctggtgcagcctggcggctctctgagactgtcttgcgccgcctccggcttcaccttctccgactactacatgtcctgggtgcgacaggcccctggcaagggcctggaatgggtgtcctccatctcccccgacgcctccaacacctactacgccgactccgtgaagggccggttcaccatctcccgggacaactccaagaacaccctgtacctgcagatgaactccctgcgggccgaggacaccgccgtgtactactgcgccaagaacctgcgggccttcgactactggggccagggcacactggtgaccgtgtcctccgcctccaccaagggcccctccgtgttccccctggccccctcctccaagtccacctccggcggcaccgccgccctgggctgcctggtgaaggactacttccccgagcccgtgaccgtgtcctggaactccggcgccctgacctccggcgtgcacaccttccccgccgtgctgcagtcctccggcctgtactccctgtcctccgtcgtgaccgtgccctcctcctccctgggcacccagacctacatctgcaacgtgaaccacaagccctccaacaccaaggtggacaagaaggtggagcccaagtcctgcgacaagacccacacctgccctccctgccccgcccccgagctgctgggcggcccctccgtgttcctgttccctcctaagcccaaggacaccctgatgatctcccggacccccgaggtgacttgcgtggtggtggacgtgtcccacgaggaccccgaggtgaagttcaactggtacgtggacggcgtggaggtgcacaacgccaagaccaagccccgggaggagcagtacaactccacctaccgggtggtgtccgtgctgaccgtgctgcaccaggactggctgaacggcaaggagtacaagtgcaaggtgtccaacaaggccctgcccgcccccatcgagaagaccatctccaaggccaagggccagccccgggagccccaggtgtacaccctgcccccctcccgggaggagatgaccaagaaccaggtgtccctgacctgcctggtgaagggcttctacccctccgacatcgccgtggagtgggagtccaacggccagcccgagaacaactacaagaccaccccccccgtgctggactccgacggctccttcttcctgtactccaagctgaccgtggacaagtcccggtggcagcagggcaacgtgttctcctgctccgtgatgcacgaggccctgcacaaccactacacccagaagtccctgtccctgtcccccggcaag

SEQ ID NO: 103 - DNA, 1353 bp, synthetic construct
  source 1..1353: mol_type = other DNA; note = Heavy chain coding gene
gaggtgcagctgctggagtccggcggcggcctggtgcagcccggcggctccctgcggctgtcctgcgccgcctccggcttcaccttctccaactacgacatgtcctgggtgcggcaggcccccggcaagggcctggagtgggtgtccgccatctaccactccggctcctccaagtactacgccgactccgtgaagggccggttcaccatctcccgggacaactccaagaacaccctgtacctgcagatgaactccctgcgggccgaggacaccgccgtgtactactgcgcccggggcggcaacgccgcctgggacaccggcttcgactactggggccagggcaccctggtgaccgtgtcctccgcctccaccaagggcccctccgtgttccccctggccccctcctccaagtccacctccggcggcaccgccgccctgggctgcctggtgaaggactacttccccgagcccgtgaccgtgtcctggaactccggcgccctgacctccggcgtgcacaccttccccgccgtgctgcagtcctccggcctgtactccctgtcctccgtcgtgaccgtgccctcctcctccctgggcacccagacctacatctgcaacgtgaaccacaagccctccaacaccaaggtggacaagaaggtggagcccaagtcctgcgacaagacccacacctgccctccctgccccgcccccgagctgctgggcggcccctccgtgttcctgttccctcctaagcccaaggacaccctgatgatctcccggacccccgaggtgacttgcgtggtggtggacgtgtcccacgaggaccccgaggtgaagttcaactggtacgtggacggcgtggaggtgcacaacgccaagaccaagccccgggaggagcagtacaactccacctaccgggtggtgtccgtgctgaccgtgctgcaccaggactggctgaacggcaaggagtacaagtgcaaggtgtccaacaaggccctgcccgcccccatcgagaagaccatctccaaggccaagggccagccccgggagccccaggtgtacaccctgcccccctcccgggaggagatgaccaagaaccaggtgtccctgacctgcctggtgaagggcttctacccctccgacatcgccgtggagtgggagtccaacggccagcccgagaacaactacaagaccaccccccccgtgctggactccgacggctccttcttcctgtactccaagctgaccgtggacaagtcccggtggcagcagggcaacgtgttctcctgctccgtgatgcacgaggccctgcacaaccactacacccagaagtccctgtccctgtcccccggcaag

SEQ ID NO: 104 - protein, 4 aa, synthetic construct
CVIM

SEQ ID NO: 105 - protein, 4 aa, synthetic construct
CVLL

SEQ ID NO: 106 - protein, 11 aa, synthetic construct
GGGGGGGCVIM